European Patent Specification EP 3 360 961 B1, published November 22, 2023. Title: METHOD FOR PREPARING GENE-MODIFIED T CELLS EXPRESSING CHIMERIC ANTIGEN RECEPTOR. Applicant: NATIONAL UNIVERSITY CORPORATION NAGOYA UNIVERSITY SHINSHU UNIVERSITY. The sequence listing filed with the application follows.

SEQUENCE LISTING (9 sequences)

SEQ ID NO: 1 - DNA, 6438 bp, Artificial Sequence
  pIRII-CAR.CD19.28z
  misc_feature (30)..(86): Leader
  misc_feature (87)..(416): VL
  misc_feature (486)..(833): VH
  misc_feature (867)..(1562): CH2CH3
  misc_feature (1575)..(1778): CD28
  misc_feature (1779)..(2117): CD3 zeta
  misc_feature (2850)..(3085): 3' IR
  misc_feature (5031)..(5341): 5' IR
tcgagctcaagcttcgaattcgaatggccatggagtttgggctgagctggctttttcttgtggctattttaaaaggtgtccagtgctctagagacatccagatgacacagactacatcctccctgtctgcctctctgggagacagagtcaccatcagttgcagggcaagtcaggacattagtaaatatttaaattggtatcagcaaaaaccagatggaactgttaaactcctgatctaccatacatcaagattacactcaggagtcccatcaaggttcagtggcagtgggtctggaacagattattctctcaccattagcaacctggagcaagaagatattgccacttacttttgccaacagggtaatacgcttccgtacacgttcggaggggggaccaagctggagctgaaacgtggtggtggtggttctggtggtggtggttctggcggcggcggctccggtggtggtggatccgaggtgcagctgcagcagtctggacctggcctggtggcgccctcacagagcctgtccgtcacatgcactgtctcaggggtctcattacccgactatggtgtaagctggattcgccagcctccacgaaagggtctggagtggctgggagtaatatggggtagtgaaaccacatactataattcagctctcaaatccagactgaccatcatcaaggacaactccaagagccaagttttcttaaaaatgaacagtctgcaaactgatgacacagccatttactactgtgccaaacattattactacggtggtagctatgctatggactactggggccaagggaccacggtcaccgtctcctcgtacgtcaccgtctcttcacaggatcccgccgagcccaaatctcctgacaaaactcacacatgcccaccgtgcccagcacctgaactcctggggggaccgtcagtcttcctcttccccccaaaacccaaggacaccctcatgatctcccggacccctgaggtcacatgcgtggtggtggacgtgagccacgaagaccctgaggtcaagttcaactggtacgtggacggcgtggaggtgcataatgccaagacaaagccgcgggaggagcagtacaacagcacgtaccgtgtggtcagcgtcctcaccgtcctgcaccaggactggctgaatggcaaggagtacaagtgcaaggtctccaacaaagccctcccagcccccatcgagaaaaccatctccaaagccaaagggcagccccgagaaccacaggtgtacaccctgcccccatcccgggatgagctgaccaagaaccaggtcagcctgacctgcctggtcaaaggcttctatcccagcgacatcgccgtggagtgggagagcaatgggcaaccggagaacaactacaagaccacgcctcccgtgctggactccgacggctccttcttcctctacagcaagctcaccgtggacaagagcaggtggcagcaggggaacgtcttctcatgctccgtgatgcatgaggctctgcacaaccactacacgcagaagagcctctccctgtctccgggtaaaaaagatcccaaattttgggtgctggtggtggttggtggagtcctggcttgctatagcttgctagtaacagtggcctttattattttctgggtgaggagtaagaggagcaggctcctgcacagtgactacatgaacatgactccccgccgccccgggcccacccgcaagcattaccagccctatgccccaccacgcgacttcgcagcctatcgctccagagtgaagttcagcaggagcgcagacgcccccgcgtaccagcagggccagaaccagctctataacgagctcaatctaggacgaagagaggagtacgatgttttggacaagagacgtggccgggaccctgagatggggggaaagccgagaaggaagaaccctcaggaaggcctgtacaatgaactgcagaaagataagatggcggaggcctacagtgagattgggatgaaaggcgagcgccggaggggcaaggggcacgatggcctttaccagggtctcagtacagccaccaaggacacctacgacgcccttcacatgcaggccctgcctcctcgctaagcatgctagctatagttctagaggtaccggttgttaacgttagccggctacgtatactccggaatattaataggcctaggatgcatatggcggccgcttccctttagtgagggttaatgcttcgagcagacatgataagatacattgatgagtttggacaaaccacaactagaatgcagtgaaaaaaatgctttatttgtgaaatttgtgatgctattgctttatttgtaaccattataagctgcaataaacaagttaacaacaacaattgcattcattttatgtttcaggttcagggggagatgtgggaggttttttaaagcaagtaaaacctctacaaatgtggtaaaatccgataaggatcgatccgggctggcgtaatagcgaagaggcccgcaccgatcgcccttcccaacagttgcgcagcctgaatggcgaatggacgcgccctgtagcggcgcattaagcgcggcgggtgtggtggttacgcgcagcgtgaccgctacacttgccagcgccctagcgcccgctcctttcgctttcttcccttcctttctcgccacgttcgcccgatagcgataaggatccgcgtatggtgcactctcagtacaatctgctctgatgccgcatagttaagccagccccgacacccgccaacacccgctgacgcgccctgacgggcttgtctgctcccggcatccgcttacagacaagctgtgaccgtctccgggattttgttactttatagaagaaattttgagtttttgtttttttttaataaataaataaacataaataaattgtttgttgaatttattattagtatgtaagtgtaaatataataaaacttaatatctattcaaattaataaataaacctcgatatacagaccgataaaacacatgcgtcaattttacgcatgattatctttaacgtacgtcacaatatgattatctttctagggttaatccgggagctgcatgtgtcagaggttttcaccgtcatcaccgaaacgcgcgagacgaaagggcctcgtgatacgcctatttttataggttaatgtcatgataataatggtttcttagacgtcaggtggcacttttcggggaaatgtgcgcggaacccctatttgtttatttttctaaatacattcaaatatgtatccgctcatgagacaataaccctgataaatgcttcaataatattgaaaaaggaagagtatgagtattcaacatttccgtgtcgcccttattcccttttttgcggcattttgccttcctgtttttgctcacccagaaacgctggtgaaagtaaaagatgctgaagatcagttgggtgcacgagtgggttacatcgaactggatctcaacagcggtaagatccttgagagttttcgccccgaagaacgttttccaatgatgagcacttttaaagttctgctatgtggcgcggtattatcccgtattgacgccgggcaagagcaactcggtcgccgcatacactattctcagaatgacttggttgagtactcaccagtcacagaaaagcatcttacggatggcatgacagtaagagaattatgcagtgctgccataaccatgagtgataacactgcggccaacttacttctgacaacgatcggaggaccgaaggagctaaccgcttttttgcacaacatgggggatcatgtaactcgccttgatcgttgggaaccggagctgaatgaagccataccaaacgacgagcgtgacaccacgatgcctgtagcaatggcaacaacgttgcgcaaactattaactggcgaactacttactctagcttcccggcaacaattaatagactggatggaggcggataaagttgcaggaccacttctgcgctcggcccttccggctggctggtttattgctgataaatctggagccggtgagcgtgggtctcgcggtatcattgcagcactggggccagatggtaagccctcccgtatcgtagttatctacacgacggggagtcaggcaactatggatgaacgaaatagacagatcgctgagataggtgcctcactgattaagcattggtaactgtcagaccaagtttactcatatatactttagattgatttaaaacttcatttttaatttaaaaggatctaggtgaagatcctttttgataatctcatgaccaaaatcccttaacgtgagttttcgttccactgagcgtcagaccccgtagaaaagatcaaaggatcttcttgagatcctttttttctgcgcgtaatctgctgcttgcaaacaaaaaaaccaccgctaccagcggtggtttgtttgccggatcaagagctaccaactctttttccgaaggtaactggcttcagcagagcgcagataccaaatactgttcttctagtgtagccgtagttaggccaccacttcaagaactctgtagcaccgcctacatacctcgctctgctaatcctgttaccagtggctgctgccagtggcgataagtcgtgtcttaccgggttggactcaagacgatagttaccggataaggcgcagcggtcgggctgaacggggggttcgtgcacacagcccagcttggagcgaacgacctacaccgaactgagatacctacagcgtgagctatgagaaagcgccacgcttcccgaagggagaaaggcggacaggtatccggtaagcggcagggtcggaacaggagagcgcacgagggagcttccagggggaaacgcctggtatctttatagtcctgtcgggtttcgccacctctgacttgagcgtcgatttttgtgatgctcgtcaggggggcggagcctatggaaaaacgccagcaacgcggcctttttacggttcctggccttttgctggccttttgctcacatggctcgacagatctttaaccctagaaagatagtctgcgtaaaattgacgcatgcattcttgaaatattgctctctctttctaaatagcgcgaatccgtcgctgtgcatttaggacatctcagtcgccgcttggagctcccgtgaggcgtgcttgtcaatgcggtaagtgtcactgattttgaactataacgaccgcgtgagtcaaaatgacgcatgattatcttttacgtgacttttaagatttaactcatacgataattatattgttatttcatgttctacttacgtgataacttattatatatatattttcttgttatagataagatcttcaatattggccattagccatattattcattggttatatagcataaatcaatattggctattggccattgcatacgttgtatctatatcataatatgtacatttatattggctcatgtccaatatgaccgccatgttggcattgattattgactagttattaatagtaatcaattacggggtcattagttcatagcccatatatggagttccgcgttacataacttacggtaaatggcccgcctggctgaccgcccaacgacccccgcccattgacgtcaataatgacgtatgttcccatagtaacgccaatagggactttccattgacgtcaatgggtggagtatttacggtaaactgcccacttggcagtacatcaagtgtatcatatgccaagtccgccccctattgacgtcaatgacggtaaatggcccgcctggcattatgcccagtacatgaccttacgggactttcctacttggcagtacatctacgtattagtcatcgctattaccatggtgatgcggttttggcagtacaccaatgggcgtggatagcggtttgactcacggggatttccaagtctccaccccattgacgtcaatgggagtttgttttggcaccaaaatcaacgggactttccaaaatgtcgtaacaactgcgatcgcccgccccgttgacgcaaatgggcggtaggcgtgtacggtgggaggtctatataagcagagctcgtttagtgaaccgtcagatcactagaagctttattgcggtagtttatcacagttaaattgctaacgcagtcagtgcttctgacacaacagtctcgaacttaagctgcagtgactctcttaaggtagccttgcagaagttggtcgtgaggcactgggcaggtaagtatcaaggttacaagacaggtttaaggagaccaatagaaactgggcttgtcgagacagagaagactcttgcgtttctgataggcacctattggtcttactgacatccactttgcctttctctccacaggtgtccactcccagttcaattacagctcttaaggctagagtacttaatacgactcactataggctagcc

SEQ ID NO: 2 - protein, 19 aa, Artificial Sequence
  Leader
MEFGLSWLFLVAILKGVQC

SEQ ID NO: 3 - protein, 110 aa, Artificial Sequence
  VL
SRDIQMTQTTSSLSASLGDRVTISCRASQDISKYLNWYQQKPDGTVKLLIYHTSRLHSGVPSRFSGSGSGTDYSLTISNLEQEDIATYFCQQGNTLPYTFGGGTKLELKR

SEQ ID NO: 4 - protein, 116 aa, Artificial Sequence
  VH
LQQSGPGLVAPSQSLSVTCTVSGVSLPDYGVSWIRQPPRKGLEWLGVIWGSETTYYNSALKSRLTIIKDNSKSQVFLKMNSLQTDDTAIYYCAKHYYYGGSYAMDYWGQGTTVTVS

SEQ ID NO: 5 - protein, 232 aa, Artificial Sequence
  CH2CH3
EPKSPDKTHTCPPCPAPELLGGPSVFLFPPKPKDTLMISRTPEVTCVVVDVSHEDPEVKFNWYVDGVEVHNAKTKPREEQYNSTYRVVSVLTVLHQDWLNGKEYKCKVSNKALPAPIEKTISKAKGQPREPQVYTLPPSRDELTKNQVSLTCLVKGFYPSDIAVEWESNGQPENNYKTTPPVLDSDGSFFLYSKLTVDKSRWQQGNVFSCSVMHEALHNHYTQKSLSLSPGK

SEQ ID NO: 6 - protein, 68 aa, Artificial Sequence
  CD28
FWVLVVVGGVLACYSLLVTVAFIIFWVRSKRSRLLHSDYMNMTPRRPGPTRKHYQPYAPPRDFAAYRS

SEQ ID NO: 7 - protein, 112 aa, Artificial Sequence
  CD3zeta
RVKFSRSADAPAYQQGQNQLYNELNLGRREEYDVLDKRRGRDPEMGGKPRRKNPQEGLYNELQKDKMAEAYSEIGMKGERRRGKGHDGLYQGLSTATKDTYDALHMQALPPR

SEQ ID NO: 8 - DNA, 5413 bp, Artificial Sequence
  pCMV-pigBac
  misc_feature (826)..(2610): piggyBac
gaattcgagcttgcatgcctgcaggtcgttacataacttacggtaaatggcccgcctggctgaccgcccaacgacccccgcccattgacgtcaataatgacgtatgttcccatagtaacgccaatagggactttccattgacgtcaatgggtggagtatttacggtaaactgcccacttggcagtacatcaagtgtatcatatgccaagtacgccccctattgacgtcaatgacggtaaatggcccgcctggcattatgcccagtacatgaccttatgggactttcctacttggcagtacatctacgtattagtcatcgctattaccatggtgatgcggttttggcagtacatcaatgggcgtggatagcggtttgactcacggggatttccaagtctccaccccattgacgtcaatgggagtttgttttggcaccaaaatcaacgggactttccaaaatgtcgtaacaactccgccccattgacgcaaatgggcggtaggcgtgtacggtgggaggtctatataagcagagctcgtttagtgaaccgtcagatcgcctggagacgccatccacgctgttttgacctccatagaagacaccgggaccgatccagcctccggactctagaggatccggtactcgaggaactgaaaaaccagaaagttaactggtaagtttagtctttttgtcttttatttcaggtcccggatccggtggtggtgcaaatcaaagaactgctcctcagtggatgttgcctttacttctaggcctgtacggaagtgttacttctgctctaaaagctgcggaattgtacccgcggataaaatgggtagttctttagacgatgagcatatcctctctgctcttctgcaaagcgatgacgagcttgttggtgaggattctgacagtgaaatatcagatcacgtaagtgaagatgacgtccagagcgatacagaagaagcgtttatagatgaggtacatgaagtgcagccaacgtcaagcggtagtgaaatattagacgaacaaaatgttattgaacaaccaggttcttcattggcttctaacagaatcttgaccttgccacagaggactattagaggtaagaataaacattgttggtcaacttcaaagtccacgaggcgtagccgagtctctgcactgaacattgtcagatctcaaagaggtccgacgcgtatgtgccgcaatatatatgacccacttttatgcttcaaactattttttactgatgagataatttcggaaattgtaaaatggacaaatgctgagatatcattgaaacgtcgggaatctatgacaggtgctacatttcgtgacacgaatgaagatgaaatctatgctttctttggtattctggtaatgacagcagtgagaaaagataaccacatgtccacagatgacctctttgatcgatctttgtcaatggtgtacgtctctgtaatgagtcgtgatcgttttgattttttgatacgatgtcttagaatggatgacaaaagtatacggcccacacttcgagaaaacgatgtatttactcctgttagaaaaatatgggatctctttatccatcagtgcatacaaaattacactccaggggctcatttgaccatagatgaacagttacttggttttagaggacggtgtccgtttaggatgtatatcccaaacaagccaagtaagtatggaataaaaatcctcatgatgtgtgacagtggtacgaagtatatgataaatggaatgccttatttgggaagaggaacacagaccaacggagtaccactcggtgaatactacgtgaaggagttatcaaagcctgtgcacggtagttgtcgtaatattacgtgtgacaattggttcacctcaatccctttggcaaaaaacttactacaagaaccgtataagttaaccattgtgggaaccgtgcgatcaaacaaacgcgagataccggaagtactgaaaaacagtcgctccaggccagtgggaacatcgatgttttgttttgacggaccccttactctcgtctcatataaaccgaagccagctaagatggtatacttattatcatcttgtgatgaggatgcttctatcaacgaaagtaccggtaaaccgcaaatggttatgtattataatcaaactaaaggcggagtggacacgctagaccaaatgtgttctgtgatgacctgcagtaggaagacgaataggtggcctatggcattattgtacggaatgataaacattgcctgcataaattcttttattatatacagccataatgtcagtagcaagggagaaaaggttcaaagtcgcaaaaaatttatgagaaacctttacatgagcctgacgtcatcgtttatgcgtaagcgtttagaagctcctactttgaagagatatttgcgcgataatatctctaatattttgccaaatgaagtgcctggtacatcagatgacagtactgaagagccagtaatgaaaaaacgtacttactgtacttactgcccctctaaaataaggcgaaaggcaaatgcatcgtgcaaaaaatgcaaaaaagttatttgtcgagagcataatattgatatgtgccaaagttgtttctgactgactaataagtataatttgtttctattatgtataagttaagctaattaggatctaagctgcaataaacaagttaacaacaacaattgcattcattttatgtttcaggttcagggggaggtgtgggaggttttttcggatcctctagagtcgacctgcaggcatgcaagcttggcgtaatcatggtcatagctgtttcctgtgtgaaattgttatccgctcacaattccacacaacatacgagccggaagcataaagtgtaaagcctggggtgcctaatgagtgagctaactcacattaattgcgttgcgctcactgcccgctttccagtcgggaaacctgtcgtgccagctgcattaatgaatcggccaacgcgcggggagaggcggtttgcgtattgggcgctcttccgcttcctcgctcactgactcgctgcgctcggtcgttcggctgcggcgagcggtatcagctcactcaaaggcggtaatacggttatccacagaatcaggggataacgcaggaaagaacatgtgagcaaaaggccagcaaaaggccaggaaccgtaaaaaggccgcgttgctggcgtttttccataggctccgcccccctgacgagcatcacaaaaatcgacgctcaagtcagaggtggcgaaacccgacaggactataaagataccaggcgtttccccctggaagctccctcgtgcgctctcctgttccgaccctgccgcttaccggatacctgtccgcctttctcccttcgggaagcgtggcgctttctcatagctcacgctgtaggtatctcagttcggtgtaggtcgttcgctccaagctgggctgtgtgcacgaaccccccgttcagcccgaccgctgcgccttatccggtaactatcgtcttgagtccaacccggtaagacacgacttatcgccactggcagcagccactggtaacaggattagcagagcgaggtatgtaggcggtgctacagagttcttgaagtggtggcctaactacggctacactagaagaacagtatttggtatctgcgctctgctgaagccagttaccttcggaaaaagagttggtagctcttgatccggcaaacaaaccaccgctggtagcggtggtttttttgtttgcaagcagcagattacgcgcagaaaaaaaggatctcaagaagatcctttgatcttttctacggggtctgacgctcagtggaacgaaaactcacgttaagggattttggtcatgagattatcaaaaaggatcttcacctagatccttttaaattaaaaatgaagttttaaatcaatctaaagtatatatgagtaaacttggtctgacagttaccaatgcttaatcagtgaggcacctatctcagcgatctgtctatttcgttcatccatagttgcctgactccccgtcgtgtagataactacgatacgggagggcttaccatctggccccagtgctgcaatgataccgcgagacccacgctcaccggctccagatttatcagcaataaaccagccagccggaagggccgagcgcagaagtggtcctgcaactttatccgcctccatccagtctattaattgttgccgggaagctagagtaagtagttcgccagttaatagtttgcgcaacgttgttgccattgctacaggcatcgtggtgtcacgctcgtcgtttggtatggcttcattcagctccggttcccaacgatcaaggcgagttacatgatcccccatgttgtgcaaaaaagcggttagctccttcggtcctccgatcgttgtcagaagtaagttggccgcagtgttatcactcatggttatggcagcactgcataattctcttactgtcatgccatccgtaagatgcttttctgtgactggtgagtactcaaccaagtcattctgagaatagtgtatgcggcgaccgagttgctcttgcccggcgtcaatacgggataataccgcgccacatagcagaactttaaaagtgctcatcattggaaaacgttcttcggggcgaaaactctcaaggatcttaccgctgttgagatccagttcgatgtaacccactcgtgcacccaactgatcttcagcatcttttactttcaccagcgtttctgggtgagcaaaaacaggaaggcaaaatgccgcaaaaaagggaataagggcgacacggaaatgttgaatactcatactcttcctttttcaatattattgaagcatttatcagggttattgtctcatgagcggatacatatttgaatgtatttagaaaaataaacaaataggggttccgcgcacatttccccgaaaagtgccacctgacgtctaagaaaccattattatcatgacattaacctataaaaataggcgtatcacgaggccctttcgtctcgcgcgtttcggtgatgacggtgaaaacctctgacacatgcagctcccggagacggtcacagcttgtctgtaagcggatgccgggagcagacaagcccgtcagggcgcgtcagcgggtgttggcgggtgtcggggctggcttaactatgcggcatcagagcagattgtactgagagtgcaccatatgcggtgtgaaataccgcacagatgcgtaaggagaaaataccgcatcaggcgccattcgccattcaggctgcgcaactgttgggaagggcgatcggtgcgggcctcttcgctattacgccagctggcgaaagggggatgtgctgcaaggcgattaagttgggtaacgccagggttttcccagtcacgacgttgtaaaacgacggccagt

SEQ ID NO: 9 - DNA, 5793 bp, Artificial Sequence
  pIRII-CAR.CD19_optimized
tcgagctcaagcttcgaattcaccatgcttctcctggtgacaagccttctgctctgtgagttaccacacccagcattcctcctgatcccagacatccagatgacacagactacatcctccctgtctgcctctctgggagacagagtcaccatcagttgcagggcaagtcaggacattagtaaatatttaaattggtatcagcaaaaaccagatggaactgttaaactcctgatctaccatacatcaagattacactcaggagtcccatcaaggttcagtggcagtgggtctggaacagattattctctcaccattagcaacctggagcaagaagatattgccacttacttttgccaacagggtaatacgcttccgtacacgttcggaggggggactaagttggaaataacaggctccacctctggatccggcaagcccggatctggcgagggatccaccaagggcgaggtgaaactgcaggagtcaggacctggcctggtggcgccctcacagagcctgtccgtcacatgcactgtctcaggggtctcattacccgactatggtgtaagctggattcgccagcctccacgaaagggtctggagtggctgggagtaatatggggtagtgaaaccacatactataattcagctctcaaatccagactgaccatcatcaaggacaactccaagagccaagttttcttaaaaatgaacagtctgcaaactgatgacacagccatttactactgtgccaaacattattactacggtggtagctatgctatggactactggggccaagggacctcagtcaccgtctcctcagcggccgcaattgaagttatgtatcctcctccttacctagacaatgagaagagcaatggaaccattatccatgtgaaagggaaacacctttgtccaagtcccctatttcccggaccttctaagcccttttgggtgctggtggtggttggtggagtcctggcttgctatagcttgctagtaacagtggcctttattattttctgggtgaggagtaagaggagcaggctcctgcacagtgactacatgaacatgactccccgccgccccgggcccacccgcaagcattaccagccctatgccccaccacgcgacttcgcagcctatcgctccagagtgaagttcagcaggagcgcagacgcccccgcgtaccagcagggccagaaccagctctataacgagctcaatctaggacgaagagaggagtacgatgttttggacaagagacgtggccgggaccctgagatggggggaaagccgagaaggaagaaccctcaggaaggcctgtacaatgaactgcagaaagataagatggcggaggcctacagtgagattgggatgaaaggcgagcgccggaggggcaaggggcacgatggcctttaccagggtctcagtacagccaccaaggacacctacgacgcccttcacatgcaggccctgccccctcgctaaggtaccggttgttaacgttagccggctacgtatactccggaatattaataggcctaggatgcatatggcggccgcttccctttagtgagggttaatgcttcgagcagacatgataagatacattgatgagtttggacaaaccacaactagaatgcagtgaaaaaaatgctttatttgtgaaatttgtgatgctattgctttatttgtaaccattataagctgcaataaacaagttaacaacaacaattgcattcattttatgtttcaggttcagggggagatgtgggaggttttttaaagcaagtaaaacctctacaaatgtggtaaaatccgataaggatcgatccgggctggcgtaatagcgaagaggcccgcaccgatcgcccttcccaacagttgcgcagcctgaatggcgaatggacgcgccctgtagcggcgcattaagcgcggcgggtgtggtggttacgcgcagcgtgaccgctacacttgccagcgccctagcgcccgctcctttcgctttcttcccttcctttctcgccacgttcgcccgatagcgataaggatccgcgtatggtgcactctcagtacaatctgctctgatgccgcatagttaagccagccccgacacccgccaacacccgctgacgcgccctgacgggcttgtctgctcccggcatccgcttacagacaagctgtgaccgtctccgggattttgttactttatagaagaaattttgagtttttgtttttttttaataaataaataaacataaataaattgtttgttgaatttattattagtatgtaagtgtaaatataataaaacttaatatctattcaaattaataaataaacctcgatatacagaccgataaaacacatgcgtcaattttacgcatgattatctttaacgtacgtcacaatatgattatctttctagggttaatccgggagctgcatgtgtcagaggttttcaccgtcatcaccgaaacgcgcgagacgaaagggcctcgtgatacgcctatttttataggttaatgtcatgataataatggtttcttagacgtcaggtggcacttttcggggaaatgtgcgcggaacccctatttgtttatttttctaaatacattcaaatatgtatccgctcatgagacaataaccctgataaatgcttcaataatattgaaaaaggaagagtatgagtattcaacatttccgtgtcgcccttattcccttttttgcggcattttgccttcctgtttttgctcacccagaaacgctggtgaaagtaaaagatgctgaagatcagttgggtgcacgagtgggttacatcgaactggatctcaacagcggtaagatccttgagagttttcgccccgaagaacgttttccaatgatgagcacttttaaagttctgctatgtggcgcggtattatcccgtattgacgccgggcaagagcaactcggtcgccgcatacactattctcagaatgacttggttgagtactcaccagtcacagaaaagcatcttacggatggcatgacagtaagagaattatgcagtgctgccataaccatgagtgataacactgcggccaacttacttctgacaacgatcggaggaccgaaggagctaaccgcttttttgcacaacatgggggatcatgtaactcgccttgatcgttgggaaccggagctgaatgaagccataccaaacgacgagcgtgacaccacgatgcctgtagcaatggcaacaacgttgcgcaaactattaactggcgaactacttactctagcttcccggcaacaattaatagactggatggaggcggataaagttgcaggaccacttctgcgctcggcccttccggctggctggtttattgctgataaatctggagccggtgagcgtgggtctcgcggtatcattgcagcactggggccagatggtaagccctcccgtatcgtagttatctacacgacggggagtcaggcaactatggatgaacgaaatagacagatcgctgagataggtgcctcactgattaagcattggtaactgtcagaccaagtttactcatatatactttagattgatttaaaacttcatttttaatttaaaaggatctaggtgaagatcctttttgataatctcatgaccaaaatcccttaacgtgagttttcgttccactgagcgtcagaccccgtagaaaagatcaaaggatcttcttgagatcctttttttctgcgcgtaatctgctgcttgcaaacaaaaaaaccaccgctaccagcggtggtttgtttgccggatcaagagctaccaactctttttccgaaggtaactggcttcagcagagcgcagataccaaatactgttcttctagtgtagccgtagttaggccaccacttcaagaactctgtagcaccgcctacatacctcgctctgctaatcctgttaccagtggctgctgccagtggcgataagtcgtgtcttaccgggttggactcaagacgatagttaccggataaggcgcagcggtcgggctgaacggggggttcgtgcacacagcccagcttggagcgaacgacctacaccgaactgagatacctacagcgtgagctatgagaaagcgccacgcttcccgaagggagaaaggcggacaggtatccggtaagcggcagggtcggaacaggagagcgcacgagggagcttccagggggaaacgcctggtatctttatagtcctgtcgggtttcgccacctctgacttgagcgtcgatttttgtgatgctcgtcaggggggcggagcctatggaaaaacgccagcaacgcggcctttttacggttcctggccttttgctggccttttgctcacatggctcgacagatctttaaccctagaaagatagtctgcgtaaaattgacgcatgcattcttgaaatattgctctctctttctaaatagcgcgaatccgtcgctgtgcatttaggacatctcagtcgccgcttggagctcccgtgaggcgtgcttgtcaatgcggtaagtgtcactgattttgaactataacgaccgcgtgagtcaaaatgacgcatgattatcttttacgtgacttttaagatttaactcatacgataattatattgttatttcatgttctacttacgtgataacttattatatatatattttcttgttatagataagatcttcaatattggccattagccatattattcattggttatatagcataaatcaatattggctattggccattgcatacgttgtatctatatcataatatgtacatttatattggctcatgtccaatatgaccgccatgttggcattgattattgactagttattaatagtaatcaattacggggtcattagttcatagcccatatatggagttccgcgttacataacttacggtaaatggcccgcctggctgaccgcccaacgacccccgcccattgacgtcaataatgacgtatgttcccatagtaacgccaatagggactttccattgacgtcaatgggtggagtatttacggtaaactgcccacttggcagtacatcaagtgtatcatatgccaagtccgccccctattgacgtcaatgacggtaaatggcccgcctggcattatgcccagtacatgaccttacgggactttcctacttggcagtacatctacgtattagtcatcgctattaccatggtgatgcggttttggcagtacaccaatgggcgtggatagcggtttgactcacggggatttccaagtctccaccccattgacgtcaatgggagtttgttttggcaccaaaatcaacgggactttccaaaatgtcgtaacaactgcgatcgcccgccccgttgacgcaaatgggcggtaggcgtgtacggtgggaggtctatataagcagagctcgtttagtgaaccgtcagatcactagaagctttattgcggtagtttatcacagttaaattgctaacgcagtcagtgcttctgacacaacagtctcgaacttaagctgcagtgactctcttaaggtagccttgcagaagttggtcgtgaggcactgggcaggtaagtatcaaggttacaagacaggtttaaggagaccaatagaaactgggcttgtcgagacagagaagactcttgcgtttctgataggcacctattggtcttactgacatccactttgcctttctctccacaggtgtccactcccagttcaattacagctcttaaggctagagtacttaatacgactcactataggctagcc